European Patent Specification EP 3 246 338 B1, published November 22, 2023. Title: Method for preparing new type of A novel recombinant anti-TNF-A chimeric monoclonal antibody preparation method and use. Applicant: SHANGHAI ZHANGJIANG BIOTECHNOLOGY CO., LTD. Application EP16734887.9. The sequence listing filed with the application follows.

SEQUENCE LISTING (4 sequences)

SEQ ID NO: 1 - DNA, 642 bp, Artificial Sequence
  light chain of a novel anti-TNF-A monoclonal antibody
gacatcctgctgacccagtctcccgccatcctgtctgtgtctcccggcgagagagtgtctttctcttgcagagcctctcagttcgtgggctcttctatccactggtaccagcagagaaccaacggctctcccagactgctgatcaagtacgcctctgagtctatgtctggcatcccctctagattctctggctctggctctggcaccgacttcaccctgtctatcaacaccgtggagtctgaggacatcgccgactactactgccagcagtctcactcttggcccttcaccttcggctctggcaccaacctggaggtgaagagaaccgtggccgccccctctgtgttcatcttccccccctctgacgagcagctgaagtctggcaccgcctctgtggtgtgcctgctgaacaacttctaccccagagaggccaaggtgcagtggaaggtggacaacgccctgcagtctggcaactctcaggagtctgtgaccgagcaggactctaaggactctacctactctctgtcttctaccctgaccctgtctaaggccgactacgagaagcacaaggtgtacgcctgcgaggtgacccaccagggcctgtcttctcccgtgaccaagtctttcaacagaggcgagtgc

SEQ ID NO: 2 - protein, 214 aa, Artificial Sequence
  light chain of a novel anti-TNF-A monoclonal antibody
DILLTQSPAILSVSPGERVSFSCRASQFVGSSIHWYQQRTNGSPRLLIKYASESMSGIPSRFSGSGSGTDFTLSINTVESEDIADYYCQQSHSWPFTFGSGTNLEVKRTVAAPSVFIFPPSDEQLKSGTASVVCLLNNFYPREAKVQWKVDNALQSGNSQESVTEQDSKDSTYSLSSTLTLSKADYEKHKVYACEVTHQGLSSPVTKSFNRGEC

SEQ ID NO: 3 - DNA, 1350 bp, Artificial Sequence
  heavy chain of a novel anti-TNF-A monoclonal antibody
gaggtgaagctggaggagtctggcggcggcctggtgcagcccggcggctctatgaagctgtcttgcgtggcctctggcttcatcttctctaaccactggatgaactgggtgagacagtctcccgagaagggcctggagtgggtggccgagatcagatctaagtctatcaactctgccacccactacgccgagtctgtgaagggcagattcaccatctctagagacgactctaagtctgccgtgtacctgcagatgaccgacctgagaaccgaggacaccggcgtgtactactgctctagaaactactacggctctacctacgactactggggccagggcaccaccctgaccgtgtcttctgcctctaccaagggcccctctgtgttccccctggccccctcttctaagtctacctctggcggcaccgccgccctgggctgcctggtgaaggactacttccccgagcccgtgaccgtgtcttggaactctggcgccctgacctctggcgtgcacaccttccccgccgtgctgcagtcttctggcctgtactctctgtcttctgtggtgaccgtgccctcttcttctctgggcacccagacctacatctgcaacgtgaaccacaagccctctaacaccaaggtggacaagaaggtggagcccaagtcttgcgacaagacccacacctgccccccctgccccgcccccgagctgctgggcggcccctctgtgttcctgttcccccccaagcccaaggacaccctgatgatctctagaacccccgaggtgacctgcgtggtggtggacgtgtctcacgaggaccccgaggtgaagttcaactggtacgtggacggcgtggaggtgcacaacgccaagaccaagcccagagaggagcagtacaactctacctacagagtggtgtctgtgctgaccgtgctgcaccaggactggctgaacggcaaggagtacaagtgcaaggtgtctaacaaggccctgcccgcccccatcgagaagaccatctctaaggccaagggccagcccagagagccccaggtgtacaccctgcccccctctagagacgagctgaccaagaaccaggtgtctctgacctgcctggtgaagggcttctacccctctgacatcgccgtggagtgggagtctaacggccagcccgagaacaactacaagaccaccccccccgtgctggactctgacggctctttcttcctgtactctaagctgaccgtggacaagtctagatggcagcagggcaacgtgttctcttgctctgtgatgcacgaggccctgcacaaccactacacccagaagtctctgtctctgtctcccggcaag

SEQ ID NO: 4 - protein, 450 aa, Artificial Sequence
  heavy chain of a novel anti-TNF-A monoclonal antibody
EVKLEESGGGLVQPGGSMKLSCVASGFIFSNHWMNWVRQSPEKGLEWVAEIRSKSINSATHYAESVKGRFTISRDDSKSAVYLQMTDLRTEDTGVYYCSRNYYGSTYDYWGQGTTLTVSSASTKGPSVFPLAPSSKSTSGGTAALGCLVKDYFPEPVTVSWNSGALTSGVHTFPAVLQSSGLYSLSSVVTVPSSSLGTQTYICNVNHKPSNTKVDKKVEPKSCDKTHTCPPCPAPELLGGPSVFLFPPKPKDTLMISRTPEVTCVVVDVSHEDPEVKFNWYVDGVEVHNAKTKPREEQYNSTYRVVSVLTVLHQDWLNGKEYKCKVSNKALPAPIEKTISKAKGQPREPQVYTLPPSRDELTKNQVSLTCLVKGFYPSDIAVEWESNGQPENNYKTTPPVLDSDGSFFLYSKLTVDKSRWQQGNVFSCSVMHEALHNHYTQKSLSLSPGK